European Patent Specification EP 4 076 002 B1, published March 25, 2026. Title: Diet Formulations. Applicant: DuPont Nutrition Biosciences APS. The sequence listing filed with the application follows.

SEQUENCE LISTING (37 sequences)

SEQ ID NO: 1 - protein, 413 aa, artificial sequence
  PHY-13594
SEAAPAGYHLDKAVILSRHGVRAPTKMTQTMRDVTPYTWPEWPVPLGYITPRGEHLVSLMGGFYRQYFQQQGLLSRDSCPTANDVYVWTDVNQRTRKTGEAFLAGLAPECDLTIHHQNDIKQVDPLFHPVKAGICSMDKTQVQQAVEKQAGMPIDKLNQHYRPELALMSNVLNFPKSPYCQRHSGEQPCDFANAFPSKLNISDDGNEVQLEGAVGLSSTLAEIFLLEYAQGMPVVAWGNIHSEQEWNDLLKLHNAQFDLMERTPYIAKHNGTPLLQTIVNALNSNTTESKLPDISPDVKILFLAGHDTNIANIGGMLGMTWTLPGQPDNTPPGGALLFELWSDKEGTQYVSVKMVYQTLAQLRNQTPLTLKEPAGSVPLKIPGCDDQTAEGYCPLDTFTRLVNQVVEPACQLP

SEQ ID NO: 2 - protein, 413 aa, artificial sequence
  PHY-10931
SETAPAGYHLDKAVILSRHGVRAPTKMTQLMRDVTPNQWPEWPVPLGYITPRGEHLVSLMGGFYRQYFQQQGLLSRDRCPTANDVYVWTDVNQRTRKTGEAFLAGLAPQCPLTIHHQSNIKVVDPLFHPLKTGICSMDKTQVQQAVEKQAGMPIDKLNQYYAPELSLMSNVLNFPKSPYCRQHSVEKPCDFAQMFPSKLNISDDGNEVQLEGAVGLSSTLAEIFLLEHAQGMPVVAWGNIHSEQEWNDLLKLHNAQFDLMERTPYIAKHNGTPLLQTIVNALNSNTTARELPDISPDNKILFLAGHDTNIANIGGMLGMTWTLPGQPDNTPPGGALLFELWSDKAGTQYVSVHMVYQTLAQLRNQTPLTLKEPAGSVPLKIPGCDDQTAEGYCPLDTFTRLVNQVVEPACQLP

SEQ ID NO: 3 - protein, 413 aa, artificial sequence
  PHY-10957
SEAAPSGYHLQKAVILSRHGVRAPTKMTQLMRDVTPYTWPEWPVPLGYITPRGEHLVSLMGGFYRQWFQQQGILSKERCPTANDVYVWTDVNQRTRKTGEAFLAGLAPKCPLTIHHQSNIKVVDPLFHPLKTGICSMDKTQVQQAVEKQAGMPIDKLNQHYRPELALMSNVLNFPKSPYCRQHSVEKPCDFANAFPSKLNITDDGNEVQLEGAVGLSSTLAEIFLLEYAQGMPVVAWGNIHSEQEWNALLKLHNAYFDLMERTPYIAKHNGTPLLQTIVNALNSNTTARELPDISPDVKILFLAGHDTNIANIAGMLGMDWTLPGQPDNTPPGGALLFELWRDKEGTQYVSVKMVYQTLAQLRNQTPLTLKEPAGSVPLKIPGCDDQTAEGYCPLVTFTRLVNQVVEPACQIP

SEQ ID NO: 4 - protein, 413 aa, artificial sequence
  PHY-11569
SETAPSGYHLDKAVILSRHGVRAPTKMTQLMRDVTPYTWPEWPVPLGYITPRGEHLVSLMGGFYRQYFQQQGLLSKDNCPTANDVYVWTDVDQRTRKTGEAFLAGLAPECDLTIHHQNNIKVVDPMFHPLKTGICSMDKTQVQQAVEKQAGMPIDKLNQHYAPELALMSAVLNFPASPYCQQHSVDKPCDFANAFPSKLNITDDGNEVQLEGAVGLSSTLAEIFLLEYAQGMPVVAWGNIHSEQEWNALLKLHNAHFDLMSRTPYIAKHNGTPLLQTIVNALNSNTTARELPDISPDNKILFLAGHDTNIANIGGMLGMDWTLPGQPDNTPPGGALLFELWRDKAGTQYVSVHMVYQTLAQLRNQTPLTLKEPAGTVPLKIPGCDDQTAEGYCPLVTFTRLVNQSVEPACQLP

SEQ ID NO: 5 - protein, 413 aa, artificial sequence
  PHY-11658
SEAAPSGYHLDKAVLLSRHGVRAPTKMTQLMRDVTPYTWPEWPVPLGYITPRGEHLVSLMGGFYRQWFQQQGLLSKDRCPTANDVYVWADVGQRTRKTGEAFLAGLAPECDLTIHHQNDIKQVDPMFHPLKAGICSMDKTQVQQAVEKQAGMPIDKLNQHYRPELALMSNVLNFPKSPYCRQHSVEKPCDFAQMFPSKLNITDDGNEVQLEGAVGLSSTLAEIFLLEYAQGMPVVAWGNIHSEQEWNDLLKLHNAQFDLMQRTPYIAKHNGTPLLQTIVNALNSNTTARELPDISPDVKILFLAGHDTNIANIGGMLGMDWTLPGQPDNTPPGGALLFERWSDKDGTQYVSVHMVYQTLAQLRNQTPLTLKEPAGTVPLKIPGCDDQTAEGYCPLVTFTRLVNQSVEPACQLP

SEQ ID NO: 6 - protein, 413 aa, artificial sequence
  PHY-11673
SEAAPSGYHLDKAVILSRHGVRAPTKMTELMRDVTPYTWPEWPVPLGYITPRGEHLVSLMGGFYRQYFQQQGLLSKDRCPTANDVYVWTDVNQRTRKTGEAFLAGLAPECPLTIHHQSNIKVVDPLFHPVKTGLCSMDKTQVQQAVEKQAGMPIDKLNDKYAPELALMSNVLNFPKSPYCRQHSVEKPCDFAQMFPSKLSIGDDGNEVQLEGAVGLSSTLAEIFLLEYAQGMPVVAWGNIHSEQEWNDLLKLHNAHFDLMERTPYIAKHNGTPLLQTIVNALNSNTTESKLPDISPSVKILFLAGHDTNIANIGGMLGMDWTLPGQPDNTPPGGALLFELWRDKDGTQYVSVHMVYQTLAQLRNQTPLTLKEPAGTVPLKIPGCDDQTAEGYCPLVTFTVLVNQSVEPACQLP

SEQ ID NO: 7 - protein, 413 aa, artificial sequence
  PHY-11680
SETAPSGYHLDKAVILSRHGVRAPTKMTQLMRDVTPYTWPEWPVPLGYITPRGEHLVSLMGGFYRQYFQQQGLLSKDNCPTANDVYVWTDVDQRTRKTGEAFLAGLAPECDLTIHHQNNIKVVDPLFHPLKTGICSMDKTQVQQAVEKQAGMPIDKLNDHYRPELSLMSNVLNFPKSPYCQRHSGEKTCDFANAFPSKLIITDDGNKVALEGAVGLSSTLAEIFLLEYAQGMPKVAWGNIHSEQEWNDLLKLHNAQFDLMERTPYIAKHNGTPLLQTIVNALNSNTTARELPDISPDVKILFLAGHDTNIANIGGMLGMDWTLPGQPDNTPPGGALLFELWRDKEGTQYVSVKMVYQTLAQLRNQTPLTLKEPAGSVPLKIPGCDDQTAEGYCPLDTFTRLVNQVVEPACQIP

SEQ ID NO: 8 - protein, 413 aa, artificial sequence
  PHY-11895
SEAAPSGYHLDKAVLLSRHGVRAPTKMTQLMRDVTPYTWPEWPVPLGYITPRGEHLVSLMGGFYRQWFQQQGLLSRDRCPTANDVYVWTDVNQRTRKTGEAFLAGLAPECDLTIHHQKNIKVVDPLFHPLKAGICSMDKTQVQQAVEKQAGMPIDKLNQHYAPELSLMSNVLNFPKSPYCQRHSGEKTCDFANAFPSKLNISDDGNEVQLEGAVGLSSTLAEIFLLEYAQGMPVVAWGNIHSEQEWNALLKLHNAHFDLMERTPYIAKHNGTPLLQTIVNALNSNTTARELPDISPSVKILFLAGHDTNIANIGGMLGMTWTLPGQPDNTPPGGALLFELWSDKAGTQYVSVHMVYQTLTQLRNQTPLTLKEPAGSVPLKIPGCDDQTAEGYCPLDTFTRLVNQVVEPACQLP

SEQ ID NO: 9 - protein, 413 aa, artificial sequence
  PHY-11932
SETAPAGYHLDKAVILSRHGVRAPTKMTQTMRDVTPYTWPEWPVPLGYITPRGEHLVSLMGGFYRQYFQQQGLLSAERCPTANDVYVWTDVNQRTRKTGEAFLAGLAPQCPLTIHHQNDIKQVDPMFHPLKAGICSMDKTQVQQAVEKQAGMPIDKLNDHYRPELSLMSNVLNFPKSPYCARHSGDKPCDFAQMMPSKLNITDDGNEVQLEGAVGLSSTLAEIFLLEYAQGMPVVAWGNIHSEQEWNALLKLHNAQFDLMERTPYIAKHNGTPLLQTIVNALNSNTTARELPDISPDVKILFLAGHDTNIANIAGMLGMTWTLPGQPDNTPPGGALLFELWSDKAGTQYVSVHMVYQTLAQLRNQTPLTLKEPAGSVPLKIPGCDDQTAEGYCPLDTFTRLVNQVVEPACQLP

SEQ ID NO: 10 - protein, 413 aa, artificial sequence
  PHY-12058
SEAAPAGYHLDKVVILSRHGVRAPTKMTQTMRDVTPYTWPEWPVPLGYITPRGEHLVSLMGGFYRQKFQQQGLLSKDRCPTANDVYVWTDVDQRTRKTGEAFLAGLAPKCPLTIHHQSNIKVVDPLFHPLKTGICSMDKTQVQQAVEKQAGMPIDKLNQHYRPELSLMSNVLNFPKSPYCAQHSGEKPCDFAQMFPSKLNISDDGNEVQLEGAVGLSSTLAEIFLLEYAQGMPVVAWGNIHSEQEWNDLLKLHNAYFDLMERTPYIAKHNGTPLLQTIVNALNSNTTARELPDISPSVKILFLAGHDTNIANIGGMLGMDWTLPGQPDNTPPGGALLFELWRDKDGTQYVSVKMVYQTLAQLRNQTPLTLKEPAGSVPLKIPGCDDQTAEGYCPLDTFTRLVNQSVEPACQIP

SEQ ID NO: 11 - protein, 413 aa, artificial sequence
  PHY-12663
SEAAPSGYHLDKVVILSRHGVRAPTKMTQLMRDVTPYTWPEWPVPLGYITPRGEHLVSLMGGFYRQWFQQQGLLSKDRCPTANDVYVWTDVNQRTRKTGEAFLAGLAPQCPLTIHHQKNIKVVDPLFHPLKTGICSMDKTQVQQAVEKQAGMPIDKLNQHYRPELALMSNVLNFPKSPYCQRHSGDEPCDFANAFPSKLNITDDGNEVQLEGAVGLSSTLAEIFLLEYAQGMPVVAWGNIHSEQEWNDLLKLHNAQFDLMERTPYIAKHNGTPLLQTIVNALNSNTTARELPDISPDNKILFLAGHDTNIANIGGMLGMDWTLPGQPDNTPPGGALLFERWRDKEGTQYVSVHMVYQTLAQLRNQTPLTLKEPAGSVPLKIPGCDDQTAEGYCPLDTFTRLVNQVVEPACQIP

SEQ ID NO: 12 - protein, 413 aa, artificial sequence
  PHY-12784
SEAAPSGYHLDKAVLLSRHGVRAPTKMTQLMRDVTPNQWPEWPVPLGYITPRGEHLVSLMGGFYRQYFQQQGILSKDSCPTANDVYVWTDVNQRTRKTGEAFLAGLAPQCPLTIHHQSDIKQVDPMFHPLKAGICSMDKTQVQQAVEKQAGMPIDKLNQYYAPELALMSNVLNFPKSPYCQRHSGEQTCDFAQMFPSKLNISDDGNEVQLEGAVGLSSTLAETFLLEYAQGMPVVAWGNIHSEQEWNALLKLHNAQFDLMQRTPYIAKHNGTPLLQTIVNALNSNTTARELPDISPSVKILFLAGHDTNIANIGGMLGMDWTLPGQPDNTPPGGALLFELWRDKEGTQYVSVHMVYQTLTQLRNQTPLTLKEPAGTVPLKIPGCDDQTAEGYCPLVTFTRLVNQVVEPACQIP

SEQ ID NO: 13 - protein, 413 aa, artificial sequence
  PHY-13177
SEAAPSGYHLDKVVILSRHGVRAPTKMTQLMRDVTPNQWPEWPVPLGYITPRGEHLVSLMGGFYRQYFQQQGLLSKDRCPTANDVYVWADVNQRTRKTGEAFLAGLAPRCDLTIHHQKDIKQVDPMFHPLKAGICSMDKTQVQQAVEKQAGMPIDKLNQHYRPELALMSNVLNFPKSPYCAQHSGEKPCDFAQMFPSKLNISDDGNEVQLEGAVGLSSTLAEIFLLEYAQGMPVVAWGNIHSEQEWNDLLKLHNAQFDLMQRTPYIAKHNGTPLLQTIVNALNSNTTARELPDISPDNKILFLAGHDTNIANIGGMLGMDWTLPGQPDNTPPGGALLFERWRDKAGTQYVSVHMVYQTLAQLRNQTPLTLKEPAGTVPLKIPGCDDQTAEGYCPLDTFTRLVNQVVEPACQLP

SEQ ID NO: 14 - protein, 413 aa, artificial sequence
  PHY-13371
SEAAPAGYHLQKAVILSRHGVRAPTKMTQTMRDVTPYTWPEWPVPLGYITPRGEHLVKLMGGFYRQYFQQQGLLSRDRCPTANDVYVWTDVNQRTRKTGEAFLAGLAPECDLTIHHQSDIKQVDPLFHPVKAGICSMDKTQVQQAVEKQAGMPIDKLNQHYRPELALMSNVLNFPKSPYCQQHSVEQPCDFANAFPSYLNISDDGNEVQLEGAVGLGSTLAEIFLLEYAQGMPVVAWGNIHSEQEWNALLKLHNAHFNLMERTPYIAKHNGTPLLQTIVNALNSNTTARELPDISPDVKILFLAGHDTNIANIGGMLGMTWTLPGQPDNTPPGGALLFELWSDKEGTQYVAVKMVYQTLAQLRNQTPLTLKEPAGTVPLKIPGCDDQTAEGYCPLDTFTRLVNQVIEPACQLP

SEQ ID NO: 15 - protein, 413 aa, artificial sequence
  PHY-13460
SEAAPSGYHLQKAVILSRHGVRAPTKMTQLMRDVTPYTWPEWPVPLGYITPRGEHLVKLMGGFYRQYFQQQGLLSRDNCPTANDVYVWTDVAQRTRKTGEAFLAGLAPECDLTVHHQNDIKQVDPLFHPVKAGICSMNKSQVQQAVEKQAGMPIDKLNQHYRPELALMSNVLNFPKSPYCQRHSGEKPCDFAQMMPSKLNISDDGNEVQLEGAVGLSSTLAEIFLLEYAQGMPVVAWGNIHSEQEWNALLKLHNAQFDLMERTPYIAKHNGTPLMQTIVNALNSNTTARELPDISPDVKILFLAGHDTNIANIAGMLGMTWTLPGQPDNTPPGGALLFELWSDKEGTQYVSVKMVYQTLAQLRNQTPLTLKEPAGTVPLKIPGCDDQTAEGYCPLDTFTRLVNQVVEPACQLP

SEQ ID NO: 16 - protein, 413 aa, artificial sequence
  PHY-13513
SEAAPSGYHLQKAVILSRHGVRAPTKMTQLMRDVTPYTWPEWPVPLGYITPRGEHLVKLMGGFYRQYFQQQGLLSRDSCPTANDVYVWTDVNQRTRKTGEAFLAGLAPGCDLTIHHQSDIKQADPLFHPVKAGICSMDKTQVQQAVEKQAGGPIETLNQRYQAELALMSSVLDFPKSPYCQRHSVDKPCDFANAFPSYLNISDDGNEVQLEGAVGLSSTLAEIFLLEYAQGMPVVAWGNIHSEQEWNALLKLHNAHFDLMERTPYIAKHNGTPLLQTIVNALNSNTTARELPDISPDVKILFLAGHDTNIANIGGMLGMTWTLPGQPDNTPPGGALLFELWRDKDGTQYVSVHMVYQTLAQLRNMTPLTLKEPAGSVPLKIPGCDDQTAEGYCPLDTFTRLVNQVVEPACQLP

SEQ ID NO: 17 - protein, 413 aa, artificial sequence
  PHY-13637
SEAAPAGYHLQKAVILSRHGVRAPTKMTQLMRDVTPYTWPEWPVPLGYITPRGEHLVSLMGGFYRQYFQQQGLLSKDNCPTANDVYVWTDVNQRTRKTGEAFLAGLAPECDLTIHHQNDIKQVDPLFHPLKAGICSMDKTQVQQAVEKQAGMPIDKLNQHYRPELALMSSVLDFPKSPYCQHHSGDQPCDFAQMFPSYLNISDDGNEVQLEGAVGLSSTLAEIFLLEYAQGMPVVAWGNIHSEQEWNDLLKLHNAYFDLMERTPYIAKHNGTPLLQTIVNALNSNTTARELPDVSPDVKILFLAGHDTNIANIGGMLGMDWTLPGQPDNTPPGGALLFELWSDKEGTQYVSVKMVYQTLAQLRNQTPLTLKEPAGSVPLKIPGCDDQTAEGYCPLDTFTRLVNQVVEPACQLP

SEQ ID NO: 18 - protein, 413 aa, artificial sequence
  PHY-13705
SEAAPAGYHLDKAVILSRHGVRAPTKMTQLMRDVTPYTWPEWPVPLGYITPRGEHLVKLMGGFYRQYFQQQGLLSRDSCPTANDVYVWTDVNQRTRKTGEAFLAGLAPECDLTIHHQSDIKQADPLFHPLKAGICSMDKTQVQQAVEKQAGMPIDKLNQHYRAELALMSNVLNFPKSPYCRQHSVEQPCDFANAFPSRLNISDDGNEVQLEGAVGLSSTLAEIFLLEYAQGMPVVAWGNIHSEQEWNDLLKLHNAYFDLMERTPYIAKHQGTPLLQTIVNALNSNTTARELPDISPDVKILFLAGHDTNIANIAGMLGMDWTLPGQPDNTPPGGALLFELWSDKEGTQYVSVKMVYQTLAQLRNQTPLTLKEPAGSVPLKIPGCDDQTAEGYCPLDTFTRLVNRVVEPACQLP

SEQ ID NO: 19 - protein, 413 aa, artificial sequence
  PHY-13713
SEAAPAGYHLQKAVILSRHGVRAPTKMTQLMRDVTPYTWPEWPVPLGYITPRGEHLVSLMGGFYRQYFQQQGLLSRDRCPTPDAVYVWTDVNQRTRKTGEAFLAGLAPECDLTIHHQNDIHQVDPLFHPVKAGICSMDKTQVQQAVEKQAGMPIDKLNQHYRPELALMSNVLNFPKSPYCQRHSVDKPCDFAQMMPSYLNISDDGNEVQLEGAVGLSSTLAEIFLLEYAQGMPVVAWGNIHSEQEWNDLLKLHNAHFDLMERTPYIAKHQGTPLLQTIVNALNSNTTESKLPDISPDVKILFLAGHDTNIANIAGMLGMTWTLPGQPDNTPPGGALLFELWRDKAGTQYVSVKMVYQTLAQLRNQTPLTLKEPAGSVPLKIPGCDDQTAEGYCPLDTFTRLVNQVVEPACQLP

SEQ ID NO: 20 - protein, 412 aa, artificial sequence
  PHY-13747
SEAAPSGYHLQKAVILSRHGVRAPTKMTQLMRDVTPYTWPEWPVPLGYITPRGEHLVSLMGGFYRQYFQQQGLLSKDNCPTANDVYVWTDVNQRTRKTGEAFLAGLAPQCDLAIHHQNDIKQVDPLFHPLKAGICSMDKTQVQQAVEKQAGMPIDKLNQHYRPELALMSNVLNFPKSPYCRRHSGEKPCDFAQMMPSKLNISDDGNEVQLEGAVGLSSTLAEIFLLEYAQGMPVVAWGNIHSEEEWNDLLKLHNAYFDLMQRTPYIAKHNGTPLMQTISNALNPNATESKLPDISPDNKILFIAGHDTNIANIGGMLGMTWTLPGQPDNTPPGGALLFELWSDKEGTQYVSVKMVYQTLAQLRNQTPLTLKEPAGTVPLKIPGCDDQTAEGYCPLDTFTRLVNQVVEPACQI

SEQ ID NO: 21 - protein, 412 aa, artificial sequence
  PHY-13779
SEAAPAGYHLQKAVILSRHGVRAPTKMTQTMRDVTPHQWPEWPVPLGYITPRGEHLVKLMGGFYRQYFQQQGLLSKDRCPTANDVYVWTDVNQRTRKTGEAFLAGLAPECDLTIHHQSDIKQVDPLFHPLKAGICSMDKTQVQQAVEKQAGMPIDELNQHYRPELALMSNVLNFPKSPYCQRHSGEQPCDFANAFPSYLNISDDGNEVQLEGAVGLSSTLAEIFLLEYAQGMPVVAWGNIHSEQEWNDLLKLHNAYFDLMQRTPYIAKHNGTPLLQTIVNALNSNTTARELPDISPDVKILFLAGHDTNIANIGGMLGMTWTLPGQPDNTPPGGALLFELWSDKAGTQYVSVHMVYQTLAQLRNMTPLTLKEPAGTVPLKIPGCDDQTAEGYCPLDTFTRLVNQVVEPACQI

SEQ ID NO: 22 - protein, 413 aa, artificial sequence
  PHY-13789
SEAAPAGYHLQKAVILSRHGVRAPTKMTQLMRDVTPYTWPEWPVPLGYITPRGEHLVKLMGGFYRQYFQQQGLLSRDNCPTPDDVYVWTDVNQRTRKTGEAFLAGLAPECDLTIHHQSDIKQVDPLFHPLKAGICSMDKTQVQQAVEKQAGMPIDKLNQHYRAELALMSNVLNFPKSPYCQRHSGEQPCDFAQMFPSYLNISDDGNEVQLEGAVGLSSTLAEIFLLEYAQGMPVVAWGNIHSEQEWNDLLKLHNAYFDLMERTPYIAKHNGTPLLQTIVNALNPNATESKLPDISPDVKILFLAGHDTNIANIGGMLGMDWTLPGQPDNTPPGGALLFELWSDKEGTQYVSVKMVYQTLAQLRNMTPLTLKEPAGSVPLKIPGCDDQTAEGYCPLDTFTRLVNQVVEPACQLP

SEQ ID NO: 23 - protein, 413 aa, artificial sequence
  PHY-13798
SEAAPAGYHLQKAVILSRHGVRAPTKMTQTMRDVTPYTWPEWPVPLGYITPRGEHLVKLMGGFYRQYFQQQGLLSKDNCPTANDVYVWTDVAQRTRKTGEAFLAGLAPECDLTIHHQNNISQVDPLFHPVKAGICSMDKTQVQQAVEKQAGMPIDKLNQHYRPELALMSNVLNFPKSPYCQRHSGEKPCDFAQMMPSKLNISDDGNEVQLEGAVGLSSTLAEIFLLEYAQGMPVVAWGNIHSEQEWNDLLKLHNAHFDLMERTPYIAKHNGTPLLQAISNALNPNTTESKLPDISPDVKILFLAGHDTNIANIGGMLGMTWTLPGQPDNTPPGGALLFELWRDKAGTQYVSVHMVYQTLAQLRNMTPLTLKEPAGSVPLKIPGCDDQTAEGYCPLDTFTRLVNQVVEPACQLP

SEQ ID NO: 24 - protein, 413 aa, artificial sequence
  PHY-13868
SDTAPAGFQLEKVVILSRHGVRAPTKMTQLMRDVTPYTWPEWPVPLGYITPRGEHLISLMGGFYRQYFQQQGLLSKDNCPTANDVYVWTDVDQRTRKTGEAFLAGLAPECDLTIHHQSDIKQADPLFHPVKAGICSMDKSQTYEAVEKQAGGPIETLNQHYRPELALMSNVLNFPKSPYCRRHSGDKTCDFANAFPSYLNISDDGNEVQLEGAVGLSSTLAEIFLLEYAQGMPVVAWGNIHSEQEWNDLLKLHNAHFDLMQRTPYIAKHQGTPLLQTIVNALNSNTTARELPDISPDVKILFLAGHDTNIANIGGMLGMTWTLPGQPDNTPPGGALLFELWSDKEGTQYVSVEMVYQTLAQLRNMTPLTLKEPAGTVPLKIPGCDDQTAEGYCPLDTFTRLVNQVVEPACQLP

SEQ ID NO: 25 - protein, 413 aa, artificial sequence
  PHY-13883
SEAAPSGYQLEKVVILSRHGVRAPTKMTQTMRDVTPYTWPEWPVPLGYITPRGEHLVKLMGGFYRQYFQQQGLLSRDNCPTANDVYVWTDVDQRTRKTGEAFLAGLAPGCDLTIHHQNNISQADPLFHPVKAGICSMDKTQVQQAVEKQAGMPIDKLNQHYRAELALMSNVLNFPKSPYCRQHSVEQPCDFANAFPSYLNISDDGNEVQLEGAVGLSSTLAEIFLLEYAQGMPVVAWGNIHSEQEWNALLKLHNAHFDLMQRTPYIAKHNGTPLLQTIVNALNSNTTARELPDISPDVKILFLAGHDTNIANIGGMLGMTWTLPGQPDNTPPGGALLFELWRDKDGTQYVSVHMVYQTLAQLRNMTPLTLKEPAGSVPLKIPGCDDQTAEGYCPLDTFTRLVNQVVEPACQLP

SEQ ID NO: 26 - protein, 413 aa, artificial sequence
  PHY-13885
SEAAPSGYHLDKAVILSRHGVRAPTKMTQLMRDVTPYTWPEWPVPLGYITPRGEHLVSLMGGFYRQYFQQQGLLSRDRCPTANDVYVWTDVNQRTRKTGEAFLAGLAPECDLTIHHQNDIKQVDPLFHPLKAGICSMDKTQVQQAVEKQAGMPIDKLNQHYRPELALMSNVLNFPKSPYCRQHSVEQPCDFANAFPSYLNISDDGNEVQLEGAVGLSSTLAEIFLLEYAQGMPVVAWGNIHSEQEWNDLLKLHNAQFDLMERTPYIAKHQGTPLLQTIVNALNSNTTESKLPDISPSVKILFLAGHDTNIANIGGMLGMTWTLPGQPDNTPPGGALLFELWSDKDGTQYVSVKMVYQTLAQLRNMTPLTLKEPAGSVPLKIPGCDDQTAEGYCPLDTFTRLVNQVVEPACQLP

SEQ ID NO: 27 - protein, 413 aa, artificial sequence
  PHY-13936
SEAAPAGYHLDKAVILSRHGVRAPTKMTQTMRDVTPYTWPEWPVPLGYITPRGEHLVKLMGGFYRQYFQQQGLLPRDSCPTANDVYVWTDVNQRTRKTGEAFLAGLAPECAITIHHQSDIKQVDPLFHPVKAGICSMDKTQVQQAVEKQAGMPIDKLNQHYRPELALMSNVLNFPKSPYCQRHSGEQPCDFANAFPSYLNISDDGNEVQLEGAVGLSSTLAEIFLLEYAQGMPVVAWGNIHSEQEWNALLKLHNAHFDLMERTPYIAKHNGTPLLQTIVNALNSNTTESKLPDISPSVKILFLAGHDTNIANIGGMLGMTWTLPGQPDNTPPGGALLFELWSDKEGTQYVSVEMVYQTLAQLRNQTPLTLKEPAGSVPLKIPGCDDQTAEGYCPLDTFTRLVNQVVEPACQLP

SEQ ID NO: 28 - protein, 412 aa, artificial sequence
  PHY-14004
AEEANGMKLQKAVILSRHGVRAPTKMTQLMRDVTPYTWPEWPVPLGYITPRGEHLVSLMGGFYRQYFQQQGLLSRDSCPTANDVYVWTDVNQRTRKTGEAFLAGLAPGCDLTIHHQNDIKQVDPLFHPLKAGICSMDKTQVQQAVEKQAGMPIDKLNQHYRPELALMSNVLNFPKSPYCQRHSGEQPCDFANMFPSYLNISDDGNEVQLEGAVGLSSTLAEIFLLEYAQGMPVVAWGNIHSEQEWNDLLKLHNAQFDLMERTPYIAKHNGTPLLQTIVNALNSNTTARELPDISPDVKILFLAGHDTNIANIAGMLGMTWTLPGQPDNTPPGGALLFELWSDKDGTQYVSVHMVYQTLAQLRNQTPLTLKEPAGSVPLKIPGCDDQTAEGYCPLDTFTRLVNQVVEPACQLP

SEQ ID NO: 29 - protein, 413 aa, artificial sequence
  PHY-14215
SEAAPAGYHLQKAVILSRHGVRAPTKMTQLMRDVTPYTWPEWPVPLGYITPRGEHLVSLMGGFYRQYFQQQGLLSRDSCPTANDVYVWTDVDQRTRKTGEAFLAGLAPGCDLAIHHQQNITQVDPLFHPLKAGICSMDKTQVQQAVEKQAGMPIDKLNQHYRPELALMSNVLNFPKSPYCRRHSGDKTCDFANAFPSYLNISDDGNKVALDGAVGLSSTLAEIFLLEYAQGMPVVAWGNIHSESQWKSLLNLHNAHFNLMQRTPYIAKHNGTPLLQTIVNALNPNATESKLPDISPDNKILFLAGHDTNIANIGGMLGMTWTLPGQPDNTPPGGALLFELWRDKEGTQYVSVEMVYQTLAQLRNQTPLTLKEPAGSVPLKIPGCDDQTAEGYCPLDTFTRLVNQVVEPACQLP

SEQ ID NO: 30 - protein, 413 aa, artificial sequence
  PHY-14256
SDTAPAGYQLDKAVILSRHGVRAPTKMTQLMRDVTPYTWPEWPVPLGYITPRGEHLVKLMGGFYRQYFQQQGLLSKDNCPTANDVYVWTDVNQRTRKTGEAFLAGLAPGCDLTIHHQNDIKQADPLFHPLKAGICSMDKTQVQQAVEKQAGMPIDKLNQHYRPELALMSNVLNFPKSPYCQRHSVDKPCDFANAFPSYLNISDDGNEVQLEGAVGLSSTLAEIFLLEYAQGMPVVAWGNIHSEQEWNDLLKLHNAYFDLMQRTPYIAKHQGTPLLQTIVNALNSNTTESKLPDISPDVKILFLAGHDTNIANIAGMLGMDWTLPGQPDNTPPGGALLFELWSDKEGTQYVSVKMVYQTLAQLRNQTPLTLKEPAGSVPLKIPGCDDQTAEGYCPLDTFTRLVNQVVEPACQLP

SEQ ID NO: 31 - protein, 412 aa, artificial sequence
  PHY-14277
SEAAPAGYHLDKAVILSRHGVRAPTKMTQLMRDVTPYTWPEWPVPLGYITPRGEHLVSLMGGFYRQYFQQQGLLPKDNCPTANDVYVWTDVNQRTRKTGEAFLAGLAPECDLTIHHQNDIKQVDPLFHPVKAGICSMDKTQVQQAVEKQAGMPIDKLNQHYRPELALMSNVLNFPKSPYCRRHSGDKTCDFANAFPSYLNISDDGNEVQLEGAVGLSSTLAEIFLLEYAQGMPVVAWGNIHSEQEWNDLLKLHNAQFDLMERTPYIAKHQGTPLLQTIVNALNSNTTESKLPDISPDVKILFLAGHDTNIANIGGMLGMTWTLPGQPDNTPPGGALLFELWSDKEGTQYVSVKMVYQTLAQLRNMTPLTLKEPAGTVPLKIPGCDDQTAEGYCPLDTFTRLVNQVVEPACQI

SEQ ID NO: 32 - protein, 412 aa, artificial sequence
  PHY-14473
AEEQNGMKLQKAVILSRHGVRAPTKMTQLMRDVTPYTWPEWPVPLGYITPRGEHLVSLMGGFYRQYFQQQGLLSRDRCPTANDVYVWTDVNQRTRKTGEAFLAGLAPECAITIHHQSDIKQVDPLFHPVKAGICSMDKTQVQQAVEKQAGMPIDKLNQHYRPELALMSNVLNFPKSPYCRHQSGDKTCDFANAFPSYLNISDDGNEVQLEGAVGLSSTLAEIFLLEYAQGMPVVAWGNIHSEQEWNDLLKLHNAQFDLMERTPYIAKHNGTPLLQTIVNALNSNTTESKLPDISPDVKILFLAGHDTNIANIGGMLGMTWTLPGQPDNTPPGGALLFELWSDKEGTQYVSVKMVYQTLAQLRNQTPLTLKEPAGSVPLKIPGCDDQTAEGYCPLDTFTRLVNQVVEPACQLP

SEQ ID NO: 33 - protein, 413 aa, artificial sequence
  PHY-14614
SEAAPSGYHLDKAVILSRHGVRAPTKMTQTMRDVTPYTWPEWPVPLGYITPRGEHLVSLMGGFYRQYFQQQGLLSRDSCPTANDVYVWTDVNQRTRKTGEAFLAGLAPGCDLTIHHQQNITQVDPLFHPVKAGICSMDKTQVQQAVEKQAGMPIDKLNQHYRPELALMSNVLNFPKSPYCQQHSVDKPCDFANMFPSYLNISDDGNEVQLEGAVGLSSTLAEIFLLEYAQGMPVVAWGNIHSEQEWNDLLKLHNAQFDLMERTPYIAKHNGTPLLQTIVNALNSNTTESKLPDISPDVKILFLAGHDTNIANIAGMLGMDWTLPGQPDNTPPGGALLFELWSDKEGTQYVSVKMVYQTLAQLRNMTPLTLKEPAGTVPLKIPGCDDQTAEGYCPLDTFTRLVNQVVEPACQLP

SEQ ID NO: 34 - protein, 413 aa, artificial sequence
  PHY-14804
SDTAPAGFQLDKAVILSRHGVRAPTKMTQTMRDVTPYTWPEWPVPLGYITPRGEHLVSLMGGFYRQYFQQQGLLPRDNCPTANDVYVWTDVDQRTRKTGEAFLAGLAPECDLTIHHQSDIKQVDPLFHPLKAGICSMDKTQVQQAVEKQAGMPIDELNQHYRAELALMSNVLNFPKSPYCQRHSGEQPCDFANAFPSYLNISDDGNEVQLEGAVGLSSTLAEIFLLEYAQGMPVVAWGNIHSEQEWNDLLKLHNAQFDLMERTPYIAKHNGTPLLQTIVNALNSNTTARELPDISPDVKILFLAGHDTNIANIGGMLGMTWTLPGQPDNTPPGGALLFELWSDKDGTQYVSVKMVYQTLAQLRNQTPLTLKEPAGSVPLKIPGCDDQTAEGYCPLDTFTRLVNQVVEPACQLP

SEQ ID NO: 35 - protein, 413 aa, artificial sequence
  PHY-14945
SEAAPAGYHLDKAVILSRHGVRAPTKMTQTMRDVTPYTWPEWPVPLGYITPRGEHLVKLMGGFYRERFQQQGLLSRDSCPTANDVYVWTDVNQRTRKTGEAFLAGLAPECAITIHHQSDIKQVDPLFHPVKAGICSMDKTQVQQAVEKQAGMPIDKLNQHYRPELALMSNVLNFPKSPYCQRHSGEQPCDFANAFPSKLNISDDGNEVQLEGAVGLSSTLAEIFLLEYAQGMPVVAWGNIHSEQEWNDLLKLHNAHFDLMERTPYIAKHNGTPLLQTIVNALNSNTTARELPDISPDVKILFLAGHDTNIANIGGMLGMTWTLPGQPDNTPPGGALLFELWSDKEGTQYVSVKMVYQTLAQLRNQTPLTLKEPAGSVPLKIPGCDDQTAEGYCPLDTFTRLVNQVVEPACQLP

SEQ ID NO: 36 - protein, 412 aa, artificial sequence
  PHY-15459
AEPQNGMKLDKAVILSRHGVRAPTKMTQTMRDVTPYTWPEWPVPLGYITPRGEHLVSLMGGFYRQYFQQQGILSKDRCPRANDVYVWTDVDQRTRKTGEAFLAGLAPQCPLTIHHQNDIKQVDPMFHPVKGGICSMDKTQVQQAVEKQAGMPIDKLNDHYRPELALMSAVLNFPASPYCQRHSGEQPCDFAQMMPSKLYITDDGNEVQLEGAVGLSSTLAEIFLLEYAQGMPVVAWGNIHSEQEWNALLKLHNAYFDLMYRTPYIAKHNGTPLLQTIVNALNSNTTARELPDISPDNRILFLAGHDTNIANIGGMLGMDWTLPGQPDNTPPGGALLFELWSDKEGTQYVSVHMVYQTLAQLRNQTPLTLQEPAGTVPLKIPSCDDQTAEGYCPLDTFTKLVNQVVEPACQIP

SEQ ID NO: 37 - protein, 413 aa, artificial sequence
  PHY-16513
SEAAPSGYHLDKAVILSRHGVRAPTKMTQTMRDVTPYTWPEWPVPLGYITPRGEHLVSLMGGFYRQYFQMQGLLSRDRCPNANDVYVWTDVDQRTRKTGEAFLRGLAPECDLTIHHQNDIKQVDPMFHPVKGGICSMDKTQVQQAVEKQAGMPIDKLNDHYRPELALMSAVLNFPASPYCQQHSVDKPCDFANAFPSKLNITDDGNEVALDGAVGLSSTLAEIFLLEYAQGMPVVAWGNIHNESQWKSLLNLHNAHFNLMHRTPYIAKHNGTPLLQTIVNALNSNTTARELPDISPSVKILFLAGHDTNIANIGGMLGMDWTLPGQPDNTPPGGALLFELWSDKDGTQYVSVKMVYQTLAQLRNQTPLTLNEPAGTVPLKIPSCDDQTAEGYCPLDTFTVLVNQVVEPACQIP